European Patent Specification EP 3 612 023 B1, published July 15, 2026. Title: METHODS FOR GENERATING GENETICALLY MODIFIED ANIMAL. Applicant: eGenesis, Inc. YANG, Luhan. The sequence listing filed with the application follows.

SEQUENCE LISTING (231 sequences)

SEQ ID NO: 1 - DNA, 22 bp, Sus scrofa
ggtaccctcctccagtacgtgg

SEQ ID NO: 2 - DNA, 23 bp, Sus scrofa
ggtcatccacgtactggaggagg

SEQ ID NO: 3 - DNA, 23 bp, Sus scrofa
ggtcatccacgtactggatgagg

SEQ ID NO: 4 - DNA, 53 bp, Sus scrofa
acactctttccctacacgacgctcttccgatctcgactgccccaagggttcaa

SEQ ID NO: 5 - DNA, 55 bp, Sus scrofa
gtgactggagttcagacgtgtgctcttccgatcttctctcctgcaaatctgggcc

SEQ ID NO: 6 - DNA, 20 bp, Sus scrofa
ctgcatgaccagggtttatg

SEQ ID NO: 7 - RNA, 90 nt, Sus scrofa
  misc_feature (1)..(6): phosphodiester bond
  misc_feature (85)..(90): phosphodiester bond
aacauggaaccuuuggcccuguucauuuuagaaaucaagucaagauacgcagaagaguagacauaaacccuggucaugcagaccucagug

SEQ ID NO: 8 - DNA, 20 bp, Sus scrofa
acctttggccctgttcattt

SEQ ID NO: 9 - DNA, 23 bp, Sus scrofa
ttcgcctcagaatagaaactcag

SEQ ID NO: 10 - DNA, 23 bp, Sus scrofa
gttaggagatggcctctgttctt

SEQ ID NO: 11 - DNA, 28 bp, Sus scrofa
  misc_signal (1)..(1): 56-FAM
  misc_signal (28)..(28): 3BHQ_1
ccaaacccttatttggtcctatagcaac

SEQ ID NO: 12 - DNA, 23 bp, Sus scrofa
gggcaagtacaaagtgatgaaac

SEQ ID NO: 13 - DNA, 23 bp, Sus scrofa
attccccagctcataccatttat

SEQ ID NO: 14 - DNA, 29 bp, Sus scrofa
  misc_signal (1)..(1): 56-FAM
  misc_signal (29)..(29): 3BHQ_1
ataagagctgctccccatcagacttagat

SEQ ID NO: 15 - DNA, 23 bp, Sus scrofa
taaatggtatgtcttggggaatg

SEQ ID NO: 16 - DNA, 23 bp, Sus scrofa
agaccgtatttggtcctatagcc

SEQ ID NO: 17 - DNA, 24 bp, Sus scrofa
  misc_signal (1)..(1): 56-FAM
  misc_signal (24)..(24): 3BHQ_1
cctggttgtttacccgagcctcca

SEQ ID NO: 18 - DNA, 20 bp, Sus scrofa
cgactgccccaagggttcaa

SEQ ID NO: 19 - DNA, 21 bp, Sus scrofa
ccgactgccccaagagttcaa

SEQ ID NO: 20 - DNA, 24 bp, Sus scrofa
  misc_signal (1)..(1): 56-FAM
cacgtactggaggagggtcacctg

SEQ ID NO: 21 - DNA, 22 bp, Sus scrofa
ccgcgatctaatgttctctttc

SEQ ID NO: 22 - DNA, 20 bp, Sus scrofa
ttcactccgaccttcaccat

SEQ ID NO: 23 - DNA, 20 bp, Sus scrofa
  misc_signal (1)..(1): 5HEX
cagccgcgtccctgagacac

SEQ ID NO: 24 - DNA, 18 bp, Sus scrofa
atgcccccgaattccaga

SEQ ID NO: 25 - DNA, 23 bp, Sus scrofa
ggttaggttgcattttcatcctt

SEQ ID NO: 26 - DNA, 23 bp, Sus scrofa
atactcccctgctaccggttagg

SEQ ID NO: 27 - DNA, 23 bp, Sus scrofa
caatgattatcgaccagtacagg

SEQ ID NO: 28 - DNA, 23 bp, Sus scrofa
acttgagagaggtcaataaaagg

SEQ ID NO: 29 - DNA, 23 bp, Sus scrofa
tgagcgccctcccgcctgaacgg

SEQ ID NO: 30 - DNA, 23 bp, Sus scrofa
aaccactttttgccttcgaatgg

SEQ ID NO: 31 - DNA, 23 bp, Sus scrofa
gatccaggtacgggaagaaccgg

SEQ ID NO: 32 - DNA, 23 bp, Sus scrofa
acctggacccgactgccccaagg

SEQ ID NO: 33 - DNA, 23 bp, Sus scrofa
cgaagccctacacagagacctgg

SEQ ID NO: 34 - DNA, 23 bp, Sus scrofa
cttcaggatccaacaccctcagg

SEQ ID NO: 35 - DNA, 23 bp, Sus scrofa
gtacgtggatgacctgcttctgg

SEQ ID NO: 36 - DNA, 23 bp, Sus scrofa
accaaacaggactgcttagaagg

SEQ ID NO: 37 - DNA, 23 bp, Sus scrofa
ctgctggaattgtctgacctagg

SEQ ID NO: 38 - DNA, 23 bp, Sus scrofa
ctacagagcctctgctaagaagg

SEQ ID NO: 39 - DNA, 23 bp, Sus scrofa
caggagagaggtaacatacttgg

SEQ ID NO: 40 - DNA, 23 bp, Sus scrofa
ggcttcctaaccggtagcagggg

SEQ ID NO: 41 - DNA, 23 bp, Sus scrofa
ctgtactggtcgataatcattgg

SEQ ID NO: 42 - DNA, 23 bp, Sus scrofa
tataagggttcgggaccgttggg

SEQ ID NO: 43 - DNA, 23 bp, Sus scrofa
caggcgggagggcgctcaagagg

SEQ ID NO: 44 - DNA, 23 bp, Sus scrofa
gtgtaatctcaggcagaagaagg

SEQ ID NO: 45 - DNA, 23 bp, Sus scrofa
gcaaaaagtggttggctagtggg

SEQ ID NO: 46 - DNA, 23 bp, Sus scrofa
tgcccggttcttcccgtacctgg

SEQ ID NO: 47 - DNA, 23 bp, Sus scrofa
cccttggggcagtcgggtccagg

SEQ ID NO: 48 - DNA, 23 bp, Sus scrofa
ggcttcgtcaaagatggtcgggg

SEQ ID NO: 49 - DNA, 23 bp, Sus scrofa
gttggatcctgaagttggccagg

SEQ ID NO: 50 - DNA, 23 bp, Sus scrofa
actggaggagggtcacctgaggg

SEQ ID NO: 51 - DNA, 23 bp, Sus scrofa
tggtggctcccgccagaagcagg

SEQ ID NO: 52 - DNA, 23 bp, Sus scrofa
tagcagaggctctgtagcctagg

SEQ ID NO: 53 - DNA, 23 bp, Sus scrofa
tacctctctcctgcaaatctggg

SEQ ID NO: 54 - DNA, 23 bp, Sus scrofa
ctgctaccggttaggaagcctgg

SEQ ID NO: 55 - DNA, 23 bp, Sus scrofa
aggcttcctaaccggtagcaggg

SEQ ID NO: 56 - DNA, 23 bp, Sus scrofa
caggcttcctaaccggtagcagg

SEQ ID NO: 57 - DNA, 23 bp, Sus scrofa
ttggtcccaggcttcctaaccgg

SEQ ID NO: 58 - DNA, 23 bp, Sus scrofa
acctctctcaagtcctgtactgg

SEQ ID NO: 59 - DNA, 23 bp, Sus scrofa
tgctaccggttaggaagcctggg

SEQ ID NO: 60 - DNA, 23 bp, Sus scrofa
ggtcgataatcattggtcccagg

SEQ ID NO: 61 - DNA, 23 bp, Sus scrofa
accagtacaggacttgagagagg

SEQ ID NO: 62 - DNA, 23 bp, Sus scrofa
ggtgcaggacatacacccaacgg

SEQ ID NO: 63 - DNA, 23 bp, Sus scrofa
cttgagagaggtcaataaaaggg

SEQ ID NO: 64 - DNA, 23 bp, Sus scrofa
agaggtcaataaaagggtgcagg

SEQ ID NO: 65 - DNA, 23 bp, Sus scrofa
ttataagggttcgggaccgttgg

SEQ ID NO: 66 - DNA, 23 bp, Sus scrofa
tcaagaggttataagggttcggg

SEQ ID NO: 67 - DNA, 23 bp, Sus scrofa
ccagttccgttcaggcgggaggg

SEQ ID NO: 68 - DNA, 23 bp, Sus scrofa
ctcaagaggttataagggttcgg

SEQ ID NO: 69 - DNA, 23 bp, Sus scrofa
gggcgctcaagaggttataaggg

SEQ ID NO: 70 - DNA, 23 bp, Sus scrofa
tgtaccagttccgttcaggcggg

SEQ ID NO: 71 - DNA, 23 bp, Sus scrofa
agggcgctcaagaggttataagg

SEQ ID NO: 72 - DNA, 23 bp, Sus scrofa
acggaactggtacacagtattgg

SEQ ID NO: 73 - DNA, 23 bp, Sus scrofa
accagttccgttcaggcgggagg

SEQ ID NO: 74 - DNA, 23 bp, Sus scrofa
gtgtaccagttccgttcaggcgg

SEQ ID NO: 75 - DNA, 23 bp, Sus scrofa
actgtgtaccagttccgttcagg

SEQ ID NO: 76 - DNA, 23 bp, Sus scrofa
ggctagtggggtgtaatctcagg

SEQ ID NO: 77 - DNA, 23 bp, Sus scrofa
ctccattcgaaggcaaaaagtgg

SEQ ID NO: 78 - DNA, 23 bp, Sus scrofa
caaaaagtggttggctagtgggg

SEQ ID NO: 79 - DNA, 23 bp, Sus scrofa
acctggatctctccattcgaagg

SEQ ID NO: 80 - DNA, 23 bp, Sus scrofa
tcgggtccaggtgagctgcccgg

SEQ ID NO: 81 - DNA, 23 bp, Sus scrofa
ggggagttcttgaacccttgggg

SEQ ID NO: 82 - DNA, 23 bp, Sus scrofa
gtgtagggcttcgtcaaagatgg

SEQ ID NO: 83 - DNA, 23 bp, Sus scrofa
ggcaaaaagtggttggctagtgg

SEQ ID NO: 84 - DNA, 23 bp, Sus scrofa
attcgaaggcaaaaagtggttgg

SEQ ID NO: 85 - DNA, 23 bp, Sus scrofa
gccttcgaatggagagatccagg

SEQ ID NO: 86 - DNA, 23 bp, Sus scrofa
gaagaaccgggcagctcacctgg

SEQ ID NO: 87 - DNA, 23 bp, Sus scrofa
cgaatggagagatccaggtacgg

SEQ ID NO: 88 - DNA, 23 bp, Sus scrofa
gaatggagagatccaggtacggg

SEQ ID NO: 89 - DNA, 23 bp, Sus scrofa
atccaggtacgggaagaaccggg

SEQ ID NO: 90 - DNA, 23 bp, Sus scrofa
cttgaacccttggggcagtcggg

SEQ ID NO: 91 - DNA, 23 bp, Sus scrofa
tcttgaacccttggggcagtcgg

SEQ ID NO: 92 - DNA, 23 bp, Sus scrofa
cggggagttcttgaacccttggg

SEQ ID NO: 93 - DNA, 23 bp, Sus scrofa
tcggggagttcttgaacccttgg

SEQ ID NO: 94 - DNA, 23 bp, Sus scrofa
gggcttcgtcaaagatggtcggg

SEQ ID NO: 95 - DNA, 23 bp, Sus scrofa
agggcttcgtcaaagatggtcgg

SEQ ID NO: 96 - DNA, 23 bp, Sus scrofa
gttggccaggtctctgtgtaggg

SEQ ID NO: 97 - DNA, 23 bp, Sus scrofa
ggagggtcacctgagggtgttgg

SEQ ID NO: 98 - DNA, 23 bp, Sus scrofa
gaagcaggtcatccacgtactgg

SEQ ID NO: 99 - DNA, 23 bp, Sus scrofa
ttctaagcagtcctgtttggtgg

SEQ ID NO: 100 - DNA, 23 bp, Sus scrofa
acagagacctggccaacttcagg

SEQ ID NO: 101 - DNA, 23 bp, Sus scrofa
ggtgaccctcctccagtacgtgg

SEQ ID NO: 102 - DNA, 23 bp, Sus scrofa
tctggcgggagccaccaaacagg

SEQ ID NO: 103 - DNA, 23 bp, Sus scrofa
aggtacgaaggcactactgctgg

SEQ ID NO: 104 - DNA, 23 bp, Sus scrofa
agttggccaggtctctgtgtagg

SEQ ID NO: 105 - DNA, 23 bp, Sus scrofa
agggtgttggatcctgaagttgg

SEQ ID NO: 106 - DNA, 23 bp, Sus scrofa
gtcatccacgtactggaggaggg

SEQ ID NO: 107 - DNA, 23 bp, Sus scrofa
tactggaggagggtcacctgagg

SEQ ID NO: 108 - DNA, 23 bp, Sus scrofa
ggtcatccacgtactggaggagg

SEQ ID NO: 109 - DNA, 23 bp, Sus scrofa
gcaggtcatccacgtactggagg

SEQ ID NO: 110 - DNA, 23 bp, Sus scrofa
cgtggatgacctgcttctggcgg

SEQ ID NO: 111 - DNA, 23 bp, Sus scrofa
gtggatgacctgcttctggcggg

SEQ ID NO: 112 - DNA, 23 bp, Sus scrofa
accttctaagcagtcctgtttgg

SEQ ID NO: 113 - DNA, 23 bp, Sus scrofa
ggactgcttagaaggtacgaagg

SEQ ID NO: 114 - DNA, 23 bp, Sus scrofa
aatctgggccttcttagcagagg

SEQ ID NO: 115 - DNA, 23 bp, Sus scrofa
ctaagaaggcccagatttgcagg

SEQ ID NO: 116 - DNA, 23 bp, Sus scrofa
catacttggggtacagtttgcgg

SEQ ID NO: 117 - DNA, 23 bp, Sus scrofa
ggcccagatttgcaggagagagg

SEQ ID NO: 118 - DNA, 23 bp, Sus scrofa
ttacctctctcctgcaaatctgg

SEQ ID NO: 119 - DNA, 23 bp, Sus scrofa
aggagagaggtaacatacttggg

SEQ ID NO: 120 - DNA, 23 bp, Sus scrofa
ggagagaggtaacatacttgggg

SEQ ID NO: 121 - DNA, 23 bp, Sus scrofa
atacttggggtacagtttgcggg

SEQ ID NO: 122 - DNA, 23 bp, Sus scrofa
ctttgccaaacccatccctgcgg

SEQ ID NO: 123 - DNA, 23 bp, Sus scrofa
gccttcagttgaataacctgtgg

SEQ ID NO: 124 - DNA, 23 bp, Sus scrofa
ggtagcaggggagtattccaagg

SEQ ID NO: 125 - DNA, 23 bp, Sus scrofa
gttcaaagattaatccaacaggg

SEQ ID NO: 126 - DNA, 23 bp, Sus scrofa
caagcctgggcagaaaccgcagg

SEQ ID NO: 127 - DNA, 23 bp, Sus scrofa
tagcaggggagtattccaagggg

SEQ ID NO: 128 - DNA, 23 bp, Sus scrofa
gatattcatcatctaattggagg

SEQ ID NO: 129 - DNA, 23 bp, Sus scrofa
aagcctgggcagaaaccgcaggg

SEQ ID NO: 130 - DNA, 23 bp, Sus scrofa
ctttgacgaagccctacacaggg

SEQ ID NO: 131 - DNA, 23 bp, Sus scrofa
tacttggggtacagtttgcgggg

SEQ ID NO: 132 - DNA, 23 bp, Sus scrofa
acagtaccccttgagtagagagg

SEQ ID NO: 133 - DNA, 23 bp, Sus scrofa
gtagcaggggagtattccaaggg

SEQ ID NO: 134 - DNA, 23 bp, Sus scrofa
ttggggtacagtttgcggggcgg

SEQ ID NO: 135 - DNA, 23 bp, Sus scrofa
cttcagttgaataacctgtgggg

SEQ ID NO: 136 - DNA, 23 bp, Sus scrofa
ttgagtagagaggctcgagaagg

SEQ ID NO: 137 - DNA, 23 bp, Sus scrofa
gcggtttctgcccaggcttgggg

SEQ ID NO: 138 - DNA, 23 bp, Sus scrofa
gttggccaggtccctgtgtaggg

SEQ ID NO: 139 - DNA, 23 bp, Sus scrofa
aaggggattggacaggaactagg

SEQ ID NO: 140 - DNA, 23 bp, Sus scrofa
tcaagatatacagtcctggttgg

SEQ ID NO: 141 - DNA, 23 bp, Sus scrofa
ttcagttgaataacctgtggggg

SEQ ID NO: 142 - DNA, 23 bp, Sus scrofa
ctgggcagaaaccgcagggatgg

SEQ ID NO: 143 - DNA, 23 bp, Sus scrofa
ttggggaaactgctccaaccagg

SEQ ID NO: 144 - DNA, 23 bp, Sus scrofa
ttggagggtcaacacagtgatgg

SEQ ID NO: 145 - DNA, 23 bp, Sus scrofa
gtattccaaggggattggacagg

SEQ ID NO: 146 - DNA, 23 bp, Sus scrofa
ctcgagcctctctactcaagggg

SEQ ID NO: 147 - DNA, 23 bp, Sus scrofa
tctcgagcctctctactcaaggg

SEQ ID NO: 148 - DNA, 23 bp, Sus scrofa
gagaggctcgagaaggaatttgg

SEQ ID NO: 149 - DNA, 23 bp, Sus scrofa
tgttcaaagattaatccaacagg

SEQ ID NO: 150 - DNA, 23 bp, Sus scrofa
tcttgatcaggctttacttgggg

SEQ ID NO: 151 - DNA, 23 bp, Sus scrofa
tggattaatctttgaacatgcgg

SEQ ID NO: 152 - DNA, 23 bp, Sus scrofa
ggagcagtttccccaagcctggg

SEQ ID NO: 153 - DNA, 23 bp, Sus scrofa
ttctcgagcctctctactcaagg

SEQ ID NO: 154 - DNA, 23 bp, Sus scrofa
tagttcctgtccaatccccttgg

SEQ ID NO: 155 - DNA, 23 bp, Sus scrofa
cgaagccctacacagggacctgg

SEQ ID NO: 156 - DNA, 23 bp, Sus scrofa
atattcatcatctaattggaggg

SEQ ID NO: 157 - DNA, 23 bp, Sus scrofa
caggaactaggatgccctgttgg

SEQ ID NO: 158 - DNA, 23 bp, Sus scrofa
ggcaaagcaagttcccccacagg

SEQ ID NO: 159 - DNA, 23 bp, Sus scrofa
tggagcagtttccccaagcctgg

SEQ ID NO: 160 - DNA, 23 bp, Sus scrofa
agaaaccgcagggatgggtttgg

SEQ ID NO: 161 - DNA, 23 bp, Sus scrofa
cccacaggttattcaactgaagg

SEQ ID NO: 162 - DNA, 23 bp, Sus scrofa
gctcaaatttcttttgaacaagg

SEQ ID NO: 163 - DNA, 23 bp, Sus scrofa
tgggcagaaaccgcagggatggg

SEQ ID NO: 164 - DNA, 23 bp, Sus scrofa
tctttgacgaagccctacacagg

SEQ ID NO: 165 - DNA, 23 bp, Sus scrofa
acagggacctggccaacttcagg

SEQ ID NO: 166 - DNA, 23 bp, Sus scrofa
ggggagtattccaaggggattgg

SEQ ID NO: 167 - DNA, 23 bp, Sus scrofa
tggagggtcaacacagtgatggg

SEQ ID NO: 168 - DNA, 23 bp, Sus scrofa
gtcgatattcatcatctaattgg

SEQ ID NO: 169 - DNA, 23 bp, Sus scrofa
catccctgcggtttctgcccagg

SEQ ID NO: 170 - DNA, 23 bp, Sus scrofa
atcttgatcaggctttacttggg

SEQ ID NO: 171 - DNA, 23 bp, Sus scrofa
ctgatcaagatatacagtcctgg

SEQ ID NO: 172 - DNA, 23 bp, Sus scrofa
tatcttgatcaggctttacttgg

SEQ ID NO: 173 - DNA, 23 bp, Sus scrofa
ttgttattcacagacacttctgg

SEQ ID NO: 174 - DNA, 23 bp, Sus scrofa
gactgatactggtgtagcactgg

SEQ ID NO: 175 - DNA, 23 bp, Sus scrofa
agttggccaggtccctgtgtagg

SEQ ID NO: 176 - DNA, 23 bp, Sus scrofa
tgcggtttctgcccaggcttggg

SEQ ID NO: 177 - DNA, 23 bp, Sus scrofa
ttggaatactcccctgctaccgg

SEQ ID NO: 178 - DNA, 23 bp, Sus scrofa
caggactgtatatcttgatcagg

SEQ ID NO: 179 - DNA, 23 bp, Sus scrofa
tggggtacagtttgcggggcggg

SEQ ID NO: 180 - DNA, 23 bp, Sus scrofa
gggtactgtctgactgatactgg

SEQ ID NO: 181 - DNA, 23 bp, Sus scrofa
ctgcggtttctgcccaggcttgg

SEQ ID NO: 182 - DNA, 42 bp, Synthetic nucleic acid
gaccattaccaagcagggtctgacaggtactgaaaggatgaa

SEQ ID NO: 183 - DNA, 42 bp, Synthetic nucleic acid
attaaacaactcagccgggtgcggtgcctctgaaaggatgaa

SEQ ID NO: 184 - DNA, 42 bp, Synthetic nucleic acid
aactgtatagtcttggataaacagttcaggtgaaaggatgaa

SEQ ID NO: 185 - DNA, 42 bp, Synthetic nucleic acid
cgtgggaaacaggggctccgcgactgcgcttgaaaggatgaa

SEQ ID NO: 186 - DNA, 42 bp, Synthetic nucleic acid
gcaaatgtctttattgtttgttgctggttttgaaaggatgaa

SEQ ID NO: 187 - DNA, 42 bp, Synthetic nucleic acid
ggagtgcagtgatctgatctccgctcatggtgaaaggatgaa

SEQ ID NO: 188 - DNA, 42 bp, Synthetic nucleic acid
ccgttcctcccaaggcgggccttgaaaggatgaaaggatgaa

SEQ ID NO: 189 - DNA, 22 bp, Sus scrofa
actctatcctataaggttgaca

SEQ ID NO: 190 - DNA, 20 bp, Sus scrofa
taggttgcattttcatcctt

SEQ ID NO: 191 - DNA, 19 bp, Sus scrofa
ggagcaaaagagcagtatg

SEQ ID NO: 192 - DNA, 20 bp, Sus scrofa
taggttgcattttcatcctt

SEQ ID NO: 193 - DNA, 20 bp, Sus scrofa
tatatggacgcattcagttg

SEQ ID NO: 194 - DNA, 20 bp, Sus scrofa
taggttgcattttcatcctt

SEQ ID NO: 195 - DNA, 19 bp, Sus scrofa
ttttcggaggattttcagg

SEQ ID NO: 196 - DNA, 20 bp, Sus scrofa
taggttgcattttcatcctt

SEQ ID NO: 197 - DNA, 20 bp, Sus scrofa
tactgcatttgataccacat

SEQ ID NO: 198 - DNA, 20 bp, Sus scrofa
taggttgcattttcatcctt

SEQ ID NO: 199 - DNA, 22 bp, Sus scrofa
gacttccgtcatttatgtaaac

SEQ ID NO: 200 - DNA, 20 bp, Sus scrofa
taggttgcattttcatcctt

SEQ ID NO: 201 - DNA, 18 bp, Sus scrofa
ctctggtcgtttcagtgg

SEQ ID NO: 202 - DNA, 20 bp, Sus scrofa
taggttgcattttcatcctt

SEQ ID NO: 203 - DNA, 18 bp, Sus scrofa
cagatgagtggagcaagg

SEQ ID NO: 204 - DNA, 20 bp, Sus scrofa
taggttgcattttcatcctt

SEQ ID NO: 205 - DNA, 19 bp, Sus scrofa
gttactgggtcagggataa

SEQ ID NO: 206 - DNA, 20 bp, Sus scrofa
taggttgcattttcatcctt

SEQ ID NO: 207 - DNA, 22 bp, Sus scrofa
ccctccatatacattttctcta

SEQ ID NO: 208 - DNA, 20 bp, Sus scrofa
taggttgcattttcatcctt

SEQ ID NO: 209 - DNA, 18 bp, Sus scrofa
gagtcccattcaccaagt

SEQ ID NO: 210 - DNA, 20 bp, Sus scrofa
taggttgcattttcatcctt

SEQ ID NO: 211 - DNA, 18 bp, Sus scrofa
acgcacaagacaaagaca

SEQ ID NO: 212 - DNA, 19 bp, Sus scrofa
ctcccacccagtttcatag

SEQ ID NO: 213 - DNA, 17 bp, Sus scrofa
cccgcaaatctcacgag

SEQ ID NO: 214 - DNA, 17 bp, Sus scrofa
cccgcaaatctcacgag

SEQ ID NO: 215 - DNA, 18 bp, Sus scrofa
gtttgacagtggtgttgt

SEQ ID NO: 216 - DNA, 20 bp, Sus scrofa
taggttgcattttcatcctt

SEQ ID NO: 217 - DNA, 20 bp, Sus scrofa
tgttgagacaatagggtgat

SEQ ID NO: 218 - DNA, 20 bp, Sus scrofa
taggttgcattttcatcctt

SEQ ID NO: 219 - DNA, 20 bp, Sus scrofa
tcatgaacaagtgctgtatt

SEQ ID NO: 220 - DNA, 20 bp, Sus scrofa
taggttgcattttcatcctt

SEQ ID NO: 221 - DNA, 21 bp, Sus scrofa
ggaatagattgtcttgggaat

SEQ ID NO: 222 - DNA, 20 bp, Sus scrofa
taggttgcattttcatcctt

SEQ ID NO: 223 - DNA, 17 bp, Sus scrofa
ggctctctggggcatct

SEQ ID NO: 224 - DNA, 17 bp, Sus scrofa
caggggcctggggaatg

SEQ ID NO: 225 - DNA, 19 bp, Sus scrofa
tgtttgagaggcagaagat

SEQ ID NO: 226 - DNA, 20 bp, Sus scrofa
taggttgcattttcatcctt

SEQ ID NO: 227 - DNA, 19 bp, Sus scrofa
aggtacttggtggtgaatg

SEQ ID NO: 228 - DNA, 20 bp, Sus scrofa
taggttgcattttcatcctt

SEQ ID NO: 229 - DNA, 22 bp, Sus scrofa
tgagtatcagtatcatttgtga

SEQ ID NO: 230 - DNA, 20 bp, Sus scrofa
taggttgcattttcatcctt

SEQ ID NO: 231 - DNA, 21 bp, Sus scrofa
tctctcctgcaaatctgggcc